European Patent Application EP 4 574 212 A1, published June 25, 2025. Title: Histone deacetylase inhibitors. Applicant: Centre National de la Recherche Scientifique. Application EP. The sequence listing filed with the application follows.

SEQUENCE LISTING (41 sequences)

SEQ ID NO: 1 - protein, 10 aa, synthetic construct
AAPGKAAPGK

SEQ ID NO: 2 - protein, 10 aa, synthetic construct
AAPGKAAPGR

SEQ ID NO: 3 - protein, 10 aa, synthetic construct
AAPGKAAPGR

SEQ ID NO: 4 - protein, 10 aa, synthetic construct
AAPGRAAPGR

SEQ ID NO: 5 - protein, 10 aa, synthetic construct
  REGION 1..10: note = peptide is circular
AAPGKAAPGK

SEQ ID NO: 6 - protein, 10 aa, synthetic construct
  REGION 1..10: note = peptide is circular
AAPGKAAPGR

SEQ ID NO: 7 - protein, 10 aa, synthetic construct
  REGION 1..10: note = peptide is circular
AAPGKAAPGR

SEQ ID NO: 8 - protein, 10 aa, synthetic construct
  REGION 1..10: note = peptide is circular
AAPGRAAPGR

SEQ ID NO: 9 - protein, 10 aa, synthetic construct
AKPGKAKPGK

SEQ ID NO: 10 - protein, 10 aa, synthetic construct
  REGION 1..10: note = peptide is circular
AKPGKAKPGK

SEQ ID NO: 11 - protein, 10 aa, synthetic construct
ARPGKAKPGK

SEQ ID NO: 12 - protein, 10 aa, synthetic construct
  REGION 1..10: note = peptide is circular
ARPGKAKPGK

SEQ ID NO: 13 - protein, 10 aa, synthetic construct
AKPGKARPGK

SEQ ID NO: 14 - protein, 10 aa, synthetic construct
  REGION 1..10: note = peptide is circular
AKPGKARPGK

SEQ ID NO: 15 - protein, 10 aa, synthetic construct
ARPGKARPGK

SEQ ID NO: 16 - protein, 10 aa, synthetic construct
  REGION 1..10: note = peptide is circular
ARPGKARPGK

SEQ ID NO: 17 - protein, 10 aa, synthetic construct
AKPGKAKPGR

SEQ ID NO: 18 - protein, 10 aa, synthetic construct
  REGION 1..10: note = peptide is circular
AKPGKAKPGR

SEQ ID NO: 19 - protein, 10 aa, synthetic construct
ARPGKAKPGR

SEQ ID NO: 20 - protein, 10 aa, synthetic construct
  REGION 1..10: note = peptide is circular
ARPGKAKPGR

SEQ ID NO: 21 - protein, 10 aa, synthetic construct
AKPGKARPGR

SEQ ID NO: 22 - protein, 10 aa, synthetic construct
  REGION 1..10: note = peptide is circular
AKPGKARPGR

SEQ ID NO: 23 - protein, 10 aa, synthetic construct
ARPGKARPGR

SEQ ID NO: 24 - protein, 10 aa, synthetic construct
  REGION 1..10: note = peptide is circular
ARPGKARPGR

SEQ ID NO: 25 - protein, 10 aa, synthetic construct
AKPGRAKPGK

SEQ ID NO: 26 - protein, 10 aa, synthetic construct
  REGION 1..10: note = peptide is circular
AKPGRAKPGK

SEQ ID NO: 27 - protein, 10 aa, synthetic construct
ARPGRAKPGK

SEQ ID NO: 28 - protein, 10 aa, synthetic construct
  REGION 1..10: note = peptide is circular
ARPGRAKPGK

SEQ ID NO: 29 - protein, 10 aa, synthetic construct
AKPGRARPGK

SEQ ID NO: 30 - protein, 10 aa, synthetic construct
  REGION 1..10: note = peptide is circular
AKPGRARPGK

SEQ ID NO: 31 - protein, 10 aa, synthetic construct
ARPGRARPGK

SEQ ID NO: 32 - protein, 10 aa, synthetic construct
  REGION 1..10: note = peptide is circular
ARPGRARPGK

SEQ ID NO: 33 - protein, 10 aa, synthetic construct
AKPGRAKPGR

SEQ ID NO: 34 - protein, 10 aa, synthetic construct
  REGION 1..10: note = peptide is circular
AKPGRAKPGR

SEQ ID NO: 35 - protein, 10 aa, synthetic construct
ARPGRAKPGR

SEQ ID NO: 36 - protein, 10 aa, synthetic construct
  REGION 1..10: note = peptide is circular
ARPGRAKPGR

SEQ ID NO: 37 - protein, 10 aa, synthetic construct
AKPGRARPGR

SEQ ID NO: 38 - protein, 10 aa, synthetic construct
  REGION 1..10: note = peptide is circular
AKPGRARPGR

SEQ ID NO: 39 - protein, 10 aa, synthetic construct
ARPGRARPGR

SEQ ID NO: 40 - protein, 10 aa, synthetic construct
  REGION 1..10: note = peptide is circular
ARPGRARPGR

SEQ ID NO: 41 - protein, 10 aa, synthetic construct
  REGION 1..10: note = peptide is circular
  VARIANT 2: note = Lysine modified by an azide group
  VARIANT 5: note = Lysine modified by an azide group
  VARIANT 7: note = Lysine modified by an azide group
  VARIANT 10: note = Lysine modified by an azide group
AKPGKAKPGK